European Patent Specification EP 3 488 870 B1, published March 20, 2024. Title: Anti-CD70 Antibody Drug Conjugates. Applicant: Ambrx, Inc. Barnett, Richard S. Knudsen, Nick Sun, Ying Biroc, Sandra Buss, Timothy Javahishvili, Tsotne Bresson, Damien Srinagesh, Shailaja Hewet, Amha Pinkstaff, Jason. The sequence listing filed with the application follows.

SEQUENCE LISTING (18 sequences)

SEQ ID NO: 1 - protein, 119 aa, Homo sapiens
  MISC_FEATURE (119)..(119): X is non-natural amino acid
EVQLVQSGAEVKKPGATVKISCKVSGYTFTDYYMNWVQQAPGKGLEWMGIINPYNGGTHYNQKFKGRVTITADTSTDTAYMELSSLRSEDTAVYYCATSGYDLYFDYWGQGTLVTVSSX

SEQ ID NO: 2 - protein, 107 aa, Homo sapiens
EIVMTQSPATLSVSPGERATLSCKASQNVGTAVAWYQQKPGQAPRLLIYSAFNRYNGIPARFSGSGPGTDFTLTISSLQSEDFAVYYCQQYSTYPLTFGGGTKVEIK

SEQ ID NO: 3 - protein, 329 aa, Homo sapiens
  MISC_FEATURE (329)..(329): X is non-natural amino acid
STKGPSVFPLAPSSKSTSGGTAALGCLVKDYFPEPVTVSWNSGALTSGVHTFPAVLQSSGLYSLSSVVTVPSSSLGTQTYICNVNHKPSNTKVDKKVEPKSCDKTHTCPPCPAPPVAGGPSVFLFPPKPKDTLMISRTPEVTCVVVDVSHEDPEVKFNWYVDGVEVHNAKTKPREEQYNSTYRVVSVLTVLHQDWLNGKEYKCKVSNKALPAPIEKTISKAKGQPREPQVYTLPPSRDELTKNQVSLTCLVKGFYPSDIAVEWESNGQPENNYKTTPPVLDSDGSFFLYSKLTVDKSRWQQGNVFSCSVMHEALHNHYTQKSLSLSPGX

SEQ ID NO: 4 - protein, 328 aa, Homo sapiens
STKGPSVFPLAPSSKSTSGGTAALGCLVKDYFPEPVTVSWNSGALTSGVHTFPAVLQSSGLYSLSSVVTVPSSSLGTQTYICNVNHKPSNTKVDKKVEPKSCDKTHTCPPCPAPELLGGPSVFLFPPKPKDTLMISRTPEVTCVVVDVSHEDPEVKFNWYVDGVEVHNAKTKPREEQYNSTYRVVSVLTVLHQDWLNGKEYKCKVSNKALPAPIEKTISKAKGQPREPQVYTLPPSRDELTKNQVSLTCLVKGFYPSDIAVEWESNGQPENNYKTTPPVLDSDGSFFLYSKLTVDKSRWQQGNVFSCSVMHEALHNHYTQKSLSLSPG

SEQ ID NO: 5 - protein, 66 aa, Homo sapiens
  MISC_FEATURE (66)..(66): X is non-natural amino acid
VDNALQSGNSQESVTEQDSKDSTYSLSSTLTLSKADYEKHKVYACEVTHQGLSSPVTKSFNRGECX

SEQ ID NO: 6 - DNA, 354 bp, Homo sapiens
gaggtgcagctggttcagtctggggccgaggtgaaaaagcctggggccaccgtgaaaatttcttgtaaagtttctggatataccttcaccgattactatatgaactgggttcagcaagcccctggaaagggactggagtggatggggataattaacccatataacggcggcacccactataaccaaaagttcaaagggagggttaccatcactgcagacaccagcaccgacaccgcttatatggagctgagtagcctgaggtccgaggatactgcagtttactattgtgcgacttccggctacgatctgtactttgactactggggccagggaaccctcgttaccgtctcctca

SEQ ID NO: 7 - DNA, 321 bp, Homo sapiens
gaaattgtgatgacacagtctccggccaccctgtctgtttctccgggggaaagagctaccctgagttgcaaagccagtcagaacgttgggaccgccgttgcctggtaccaacagaaacctggccaggccccccgtctcctcatctattccgcattcaacaggtataacggcatcccagcaaggttctccggcagtgggccagggacagacttcactctcaccatcagcagcctgcagagcgaggacttcgcagtttattattgtcagcagtacagtacctaccctctcactttcggaggaggcactaaagttgagatcaaa

SEQ ID NO: 8 - DNA, 651 bp, Homo sapiens
gcacctcccgtcgccgggggaccgtcagtcttcctcttccccccaaaacccaaggacaccctcatgatctcccggacccctgaggtcacatgcgtggtggtggacgtgagccacgaagaccctgaggtcaagttcaactggtacgtggacggcgtggaggtgcataatgccaagacaaagccgcgggaggagcagtacaacagcacgtaccgtgtggtcagcgtcctcaccgtcctgcaccaggactggctgaatggcaaggagtacaagtgcaaggtctccaacaaagccctcccagcccccatcgagaaaaccatctccaaagccaaagggcagccccgagaaccacaggtgtacaccctgcccccatcccgggatgagctgaccaagaaccaggtcagcctgacctgcctggtcaaaggcttctatcccagcgacatcgccgtggagtgggagagcaatgggcagccggagaacaactacaagaccacgcctcccgtgctggactccgacggctccttcttcctctacagcaagctcaccgtggacaagagcaggtggcagcaggggaacgtcttctcatgctccgtgatgcatgaggctctgcacaaccactacacgcagaagagcctctccctgtctccgggttga

SEQ ID NO: 9 - DNA, 324 bp, Homo sapiens
cgtacggtggctgcaccatctgtcttcatcttcccgccatctgatgagcagttgaaatctggaactgcctctgttgtgtgcctgctgaataacttctatcccagagaggccaaagtacagtggaaggtggataacgccctccaatcgggtaactcccaggagagtgtcacagagcaggacagcaaggacagcacctacagcctcagcagcaccctgacgctgagcaaagcagactacgagaaacacaaagtctacgcctgcgaagtcacccatcagggcctgagctcgcccgtcacaaagagcttcaacaggggagagtgttga

SEQ ID NO: 10 - protein, 122 aa, Homo sapiens
  MISC_FEATURE (122)..(122): X is non-natural amino acid
QVQLVQSGAEVKKPGSSVKVSCKASGYSFSDYYMNWVRQAPGQGLEWMGEINPTTGGATYNQKFKARVTITADESTSTAYMELSSLRSEDTAVYYCARSLFPANYAGFVYWGQGTLVTVSSX

SEQ ID NO: 11 - protein, 106 aa, Homo sapiens
DIQMTQSPSSLSASVGDRVTITCSASSSVSYMYWYQQKPGKAPKLLIYDTSKLASGVPSRFSGSGSGTDYTFTISSLQPEDIATYYCQQWSSYPWTFGQGTKVEIK

SEQ ID NO: 12 - protein, 108 aa, Homo sapiens
  MISC_FEATURE (108)..(108): X is non-natural amino acid
RTVAAPSVFIFPPSDEQLKSGTASVVCLLNNFYPREAKVQWKVDNALQSGNSQESVTEQDSKDSTYSLSSTLTLSKADYEKHKVYACEVTHQGLSSPVTKSFNRGECX

SEQ ID NO: 13 - DNA, 363 bp, Homo sapiens
caggtgcagctggttcagtctggggccgaggtgaaaaagcctgggtcttctgtgaaagtttcttgtaaagcaagtggatattctttcagtgattactatatgaactgggttaggcaggcccctggccaaggactcgagtggatgggggagattaacccaaccaccggcggggcaacctataaccaaaagttcaaagcaagggttaccatcactgctgacgagagcacttcaactgcttatatggagctgagcagcctgaggtccgaggataccgcagtttactattgtgcgagatccctcttccctgcaaactacgcaggcttcgtttactggggacagggaaccctggtcaccgtctcctca

SEQ ID NO: 14 - DNA, 341 bp, Homo sapiens
gatattcagatgacacagtctccgtcttctctgtctgccagtgttggggatagagttaccattacctgcagtgccagttctagtgtttcctacatgtactggtaccaacagaaacctggcaaggcccccaaactcctcatctatgacacctccaaactcgcaagtggcgttccatccaggttctccggcagtgggagtgggacagactatactttcaccatcagcagcctccagcctgaggacatcgcaacctattattgtcagcagtggagtagctacccttggactttcggacagggaacgaaagttgagatcaaacgtacggtggctgcaccatctgt

SEQ ID NO: 15 - DNA, 990 bp, Homo sapiens
tagagcaccaagggcccatcggtcttccccctggcaccctcctccaagagcacctctgggggcacagcggccctgggctgcctggtcaaggactacttccccgaaccggtgacggtgtcgtggaactcaggcgccctgaccagcggcgtgcacaccttcccggctgtcctacagtcctcaggactctactccctcagcagcgtggtgaccgtgccctccagcagcttgggcacccagacctacatctgcaacgtgaatcacaagcccagcaacaccaaggtggacaagaaagttgagcccaaatcttgtgacaaaactcacacatgcccaccgtgcccagcacctcccgtcgccgggggaccgtcagtcttcctcttccccccaaaacccaaggacaccctcatgatctcccggacccctgaggtcacatgcgtggtggtggacgtgagccacgaagaccctgaggtcaagttcaactggtacgtggacggcgtggaggtgcataatgccaagacaaagccgcgggaggagcagtacaacagcacgtaccgtgtggtcagcgtcctcaccgtcctgcaccaggactggctgaatggcaaggagtacaagtgcaaggtctccaacaaagccctcccagcccccatcgagaaaaccatctccaaagccaaagggcagccccgagaaccacaggtgtacaccctgcccccatcccgggatgagctgaccaagaaccaggtcagcctgacctgcctggtcaaaggcttctatcccagcgacatcgccgtggagtgggagagcaatgggcagccggagaacaactacaagaccacgcctcccgtgctggactccgacggctccttcttcctctacagcaagctcaccgtggacaagagcaggtggcagcaggggaacgtcttctcatgctccgtgatgcatgaggctctgcacaaccactacacgcagaagagcctctccctgtctccgggttga

SEQ ID NO: 16 - DNA, 301 bp, Homo sapiens
cttcatcttcccgccatctgatgagcagttgaaatctggaactgcctctgttgtgtgcctgctgaataacttctatcccagagaggccaaagtacagtggaaggtggataacgccctccaatcgggtaactcccaggagagtgtcacagagcaggacagcaaggacagcacctacagcctcagcagcaccctgacgctgagcaaagcagactacgagaaacacaaagtctacgcctgcgaagtcacccatcagggcctgagctcgcccgtcacaaagagcttcaacaggggagagtgttga

SEQ ID NO: 17 - protein, 118 aa, Homo sapiens
QVQLVESGGGVVQPGRSLRLSCAASGFTFSSYIMHWVRQAPGKGLEWVAVISYDGRNKYYADSVKGRFTISRDNSKNTLYLQMNSLRAEDTAVYYCARDTDGYDFDYWGQGTLVTVSS

SEQ ID NO: 18 - protein, 107 aa, Homo sapiens
EIVLTQSPATLSLSPGERATLSCRASQSVSSYLAWYQQKPGQAPRLLIYDASNRATGIPARFSGSGSGTDFTLTISSLEPEDFAVYYCQQRTNWPLTFGGGTKVEIK